European Patent Application EP 4 450 637 A1, published October 23, 2024. Title: Novel self-cleaving DNAzymes and selection process. Applicant: Technische Universitaet Muenchen. The sequence listing filed with the application follows.

SEQUENCE LISTING (47 sequences)

SEQ ID NO: 1 - DNA, 31 bp, synthetic construct
  source 1..31: mol_type = other DNA
ngyygtnyacgcyyygtcttatcggttyynn

SEQ ID NO: 2 - DNA, 32 bp, synthetic construct
  source 1..32: mol_type = other DNA
ngyygtnyacgcyyygtcttatcggttynynn

SEQ ID NO: 3 - DNA, 87 bp, synthetic construct
  source 1..87: mol_type = other DNA
cagtagactaagcacactgatacagataatannnnnnnnnnnnnnnnnnnnnnnnnnnnnntattatctgacctctacctcaccatc

SEQ ID NO: 4 - DNA, 87 bp, synthetic construct
  source 1..87: mol_type = other DNA
cagtagactaagcacactgatacagataattnnnnnnnnnnnnnnnnnnnnnnnnnnnnnnaattatctgacctctacctcaccatc

SEQ ID NO: 5 - DNA, 87 bp, synthetic construct
  source 1..87: mol_type = other DNA
cagtagactaagcacactgatacagataatcnnnnnnnnnnnnnnnnnnnnnnnnnnnnnngattatctgacctctacctcaccatc

SEQ ID NO: 6 - DNA, 87 bp, synthetic construct
  source 1..87: mol_type = other DNA
cagtagactaagcacactgatacagataatgnnnnnnnnnnnnnnnnnnnnnnnnnnnnnncattatctgacctctacctcaccatc

SEQ ID NO: 7 - DNA, 56 bp, synthetic construct
  source 1..56: mol_type = other DNA
nnnnnnnnnnnnnnnnnnnnnnnnnnnnnntattatctgacctctacctcaccatc

SEQ ID NO: 8 - DNA, 87 bp, synthetic construct
  source 1..87: mol_type = other DNA
cagtagactaagcacactgatacagataatnnnnnnnnnnnnnnnnnnnnnnnnnnnnnnnnattatctgacctctacctcaccatc

SEQ ID NO: 9 - DNA, 25 bp, synthetic construct
  source 1..25: mol_type = other DNA
cagtagactaagcacactgatacag

SEQ ID NO: 10 - DNA, 31 bp, synthetic construct
  source 1..31: mol_type = other DNA
nattatctgtatcagtgtgcttagtctactg

SEQ ID NO: 11 - DNA, 31 bp, synthetic construct
  source 1..31: mol_type = other DNA
aattatctgtatcagtgtgcttagtctactg

SEQ ID NO: 12 - DNA, 31 bp, synthetic construct
  source 1..31: mol_type = other DNA
tattatctgtatcagtgtgcttagtctactg

SEQ ID NO: 13 - DNA, 31 bp, synthetic construct
  source 1..31: mol_type = other DNA
cattatctgtatcagtgtgcttagtctactg

SEQ ID NO: 14 - DNA, 31 bp, synthetic construct
  source 1..31: mol_type = other DNA
gattatctgtatcagtgtgcttagtctactg

SEQ ID NO: 15 - DNA, 57 bp, synthetic construct
  source 1..57: mol_type = other DNA
ttttttttgcagataatggtccgccgtgttaggtgcggggtcgctgtggcattatct

SEQ ID NO: 16 - DNA, 57 bp, synthetic construct
  source 1..57: mol_type = other DNA
ttttttttgcagataatcggtactaaaacagtggtgggcgggatcgccacattatct

SEQ ID NO: 17 - DNA, 56 bp, synthetic construct
  source 1..56: mol_type = other DNA
ttttttttgcagataatgggtcgtgtacgcctcgtcttatcggttatctattatct

SEQ ID NO: 18 - DNA, 57 bp, synthetic construct
  source 1..57: mol_type = other DNA
ttttttttgcagataatcagctacagcctttacctccggtgcacggacgtattatct

SEQ ID NO: 19 - DNA, 30 bp, synthetic construct
  source 1..30: mol_type = other DNA
  misc_feature 30: note = C3 spacer which is joined to another nucleic acid
tttttttttttttttttttttttttttttt

SEQ ID NO: 20 - DNA, 56 bp, synthetic construct
  source 1..56: mol_type = other DNA
  misc_feature 1: note = C3 spacer which is joined to another nucleic acid
gatggtgaggtagaggtcagataatnnnnnnnnnnnnnnnnnnnnnnnnnnnnnnn

SEQ ID NO: 21 - DNA, 87 bp, synthetic construct
  source 1..87: mol_type = other DNA
  misc_feature 1: note = C3 spacer which is joined to another nucleic acid
gatggtgaggtagaggtcagataatnnnnnnnnnnnnnnnnnnnnnnnnnnnnnnnnattatctgtatcagtgtgcttagtctactg

SEQ ID NO: 22 - DNA, 25 bp, synthetic construct
  source 1..25: mol_type = other DNA
  misc_feature 25: note = C3 spacer joined to another nucleic acid
ttttttttttttttttttttttttt

SEQ ID NO: 23 - DNA, 25 bp, synthetic construct
  source 1..25: mol_type = other DNA
  misc_feature 1: note = C3 spacer joined to another nucleic acid
gatggtgaggtagaggtcagataat

SEQ ID NO: 24 - DNA, 31 bp, synthetic construct
  source 1..31: mol_type = other DNA
ggtcgttcacgcctcgtcttatcggttttca

SEQ ID NO: 25 - DNA, 31 bp, synthetic construct
  source 1..31: mol_type = other DNA
ggtcgttcacgccttgtcttatcggttttca

SEQ ID NO: 26 - DNA, 31 bp, synthetic construct
  source 1..31: mol_type = other DNA
ggtcgttcacgcttcgtcttatcggttttca

SEQ ID NO: 27 - DNA, 31 bp, synthetic construct
  source 1..31: mol_type = other DNA
tgtcgttcacgcctcgtcttatcggttttca

SEQ ID NO: 28 - DNA, 31 bp, synthetic construct
  source 1..31: mol_type = other DNA
ggtcgtacacgccttgtcttatcggttttca

SEQ ID NO: 29 - DNA, 31 bp, synthetic construct
  source 1..31: mol_type = other DNA
ggtcgttcacgcctcgtcttatcggttttcg

SEQ ID NO: 30 - DNA, 31 bp, synthetic construct
  source 1..31: mol_type = other DNA
ggtcgttcacgccttgtcttatcggttttcg

SEQ ID NO: 31 - DNA, 31 bp, synthetic construct; identical to SEQ ID NO: 25
  source 1..31: mol_type = other DNA

SEQ ID NO: 32 - DNA, 31 bp, synthetic construct; identical to SEQ ID NO: 27
  source 1..31: mol_type = other DNA

SEQ ID NO: 33 - DNA, 31 bp, synthetic construct
  source 1..31: mol_type = other DNA
ggctgttcacgccttgtcttatcggttttcg

SEQ ID NO: 34 - DNA, 31 bp, synthetic construct; identical to SEQ ID NO: 25
  source 1..31: mol_type = other DNA

SEQ ID NO: 35 - DNA, 31 bp, synthetic construct; identical to SEQ ID NO: 27
  source 1..31: mol_type = other DNA

SEQ ID NO: 36 - DNA, 31 bp, synthetic construct; identical to SEQ ID NO: 33
  source 1..31: mol_type = other DNA

SEQ ID NO: 37 - DNA, 31 bp, synthetic construct; identical to SEQ ID NO: 30
  source 1..31: mol_type = other DNA

SEQ ID NO: 38 - DNA, 31 bp, synthetic construct; identical to SEQ ID NO: 24
  source 1..31: mol_type = other DNA

SEQ ID NO: 39 - DNA, 31 bp, synthetic construct; identical to SEQ ID NO: 25
  source 1..31: mol_type = other DNA

SEQ ID NO: 40 - DNA, 31 bp, synthetic construct; identical to SEQ ID NO: 26
  source 1..31: mol_type = other DNA

SEQ ID NO: 41 - DNA, 31 bp, synthetic construct; identical to SEQ ID NO: 28
  source 1..31: mol_type = other DNA

SEQ ID NO: 42 - DNA, 31 bp, synthetic construct; identical to SEQ ID NO: 30
  source 1..31: mol_type = other DNA

SEQ ID NO: 43 - DNA, 32 bp, synthetic construct
  source 1..32: mol_type = other DNA
ggtcgttcacgccttgtcttatcggttcctcc

SEQ ID NO: 44 - DNA, 31 bp, synthetic construct
  source 1..31: mol_type = other DNA
ggtcgttcacgcctcgtcttatcggttttcc

SEQ ID NO: 45 - DNA, 32 bp, synthetic construct
  source 1..32: mol_type = other DNA
ggtcgttcacgcctcgtcttatcggttcctcc

SEQ ID NO: 46 - DNA, 31 bp, synthetic construct
  source 1..31: mol_type = other DNA
ggtcgttcacgccttgtcttatcggttttcc

SEQ ID NO: 47 - DNA, 31 bp, synthetic construct
  source 1..31: mol_type = other DNA
ggtcgtgtacgcctcgtcttatcggttatct